European Patent Specification EP 3 709 792 B1, published December 6, 2023. Title: PLANT PROMOTER FOR TRANSGENE EXPRESSION. Applicant: Dow AgroSciences LLC SIDORENKO, LYUDMILA LARSEN, CORY ANTHONY, GENY SREEDHARAN, SRIRAM BUTLER, HOLLY. The sequence listing filed with the application follows.

SEQUENCE LISTING (27 sequences)

SEQ ID NO: 1 - DNA, 2022 bp, Artificial Sequence
  Synthetic GmPSID2 (promoter/5'UTR and terminator joined by multiple cloning site)
caaatggtaaaagaaataaatagttcatactatttttttccaaattttgaaagactttgtgatctcttacagacacaatagcaatcaaatagagaataatcttacgataaaaaaagagaaacaaactcattaaatataataataataactaggataaaataagtttatagccaatttttgttgaatctggtttttagtctatgatatatcatgtaatttagttcctaaaatttatatgaaaaaaaatggttttagtgtatgggttcactcctcaatttttgtacttttcttaacttgagatttagaaaagacactaaaaacaagtattttataaaattctgggacaaaattgtttagtatgaaagtttggaaattagacacaagatttaataaaagtttgtagactaaaaacatattttatctactaaaagtcatcaatttttataacaattatatataattatgtttataatgtaatcttagtaattagatatataaatagataaatgagacttataataataaaaaaaacatataattaactcaagtaataacaattgagaaaaagacatagaaatgtcattcttattatatctattaattagtatacatatttctttgggttagattataattaatgaaaacaaatattagtaaaaagattaatatataataattgataacaaatattattatatttattaataggtgtattttttttactataattattatatattcattaaaaaatttaaggaagggttactaaaagaaaataaaatggttttgagaagagggggggctgatttagatgtctgatttttttaattaaactgtgaagtattcttttagctgagaaacaattctgtttttgtaattgtatttttaagggatatgaagctagctaggaagatgaataagaggtgtgagttgtaagggttgggtaagggaatatgagattgtaattggtccaaggcatatcaccttatccatatccacatccaaaatctcctactttactctctctctctctctgacaaccccaacacttgtattgtctcaagcaaccggatccacacgacaccatggtgagtagttagcttaatcacttaggtcaccgagctcgcacacaactctatcttcatcatcatcatcccccgtgcttcctttatatgctatatattctcatgtgatatcatgtacctattgtcaattttattatgccacaaatattgcttaaactctgtaccttaattttacacttctttttcgctattttggtgattattatttgtgccaactgcatggtttggattaatattgatttgcttcagcttcatccaacttatgctagagtagggaatagtgatagtcatactcaaaccaaacgaggataggttgcgtaaatagtgaaatctgaaatctcgagctgaagtgagaattttgtgatcttcagtgaattgagtattaatattttatatcaaaaaggcgcgttaaagtaagatataatcgtcagggagactgttcacgttctacaagcaatttagtcgttactgcgtgctttttaacttcagattgtgagaagggactggtcatttttttaactatattgtatgattgcatggtatgaaagtttgaaagactaaaaacatgattcaatcgtatatattgaatttgaatcaaacaataaattcgggacacattcaaattaacctctgggctgaattagtgggacgggagaatcatggtcaaccctagaagaaaaaagggcttgataagacaacggaccaggtgagccatagttcaaaattgcagcaacttaaccagcttccaaaccaaatccccagacctgaatccgctgagagtttgagtttgaggaaacttaattatgtgaatttgagtttaatagatactatatatgtactattatagtgtaaacattgttaatcagttataaattatttttatatgattttttaagtaattaatataaaaatcaagaaatatataatatacaataat

SEQ ID NO: 2 - DNA, 821 bp, Artificial Sequence
  Synthetic GmPSID2 promoter
caaatggtaaaagaaataaatagttcatactatttttttccaaattttgaaagactttgtgatctcttacagacacaatagcaatcaaatagagaataatcttacgataaaaaaagagaaacaaactcattaaatataataataataactaggataaaataagtttatagccaatttttgttgaatctggtttttagtctatgatatatcatgtaatttagttcctaaaatttatatgaaaaaaaatggttttagtgtatgggttcactcctcaatttttgtacttttcttaacttgagatttagaaaagacactaaaaacaagtattttataaaattctgggacaaaattgtttagtatgaaagtttggaaattagacacaagatttaataaaagtttgtagactaaaaacatattttatctactaaaagtcatcaatttttataacaattatatataattatgtttataatgtaatcttagtaattagatatataaatagataaatgagacttataataataaaaaaaacatataattaactcaagtaataacaattgagaaaaagacatagaaatgtcattcttattatatctattaattagtatacatatttctttgggttagattataattaatgaaaacaaatattagtaaaaagattaatatataataattgataacaaatattattatatttattaataggtgtattttttttactataattattatatattcattaaaaaatttaaggaagggttactaaaagaaaataaaatggttttgagaagagggggggctgatttagatgtctgatt

SEQ ID NO: 3 - DNA, 248 bp, Glycine max
tttttaattaaactgtgaagtattcttttagctgagaaacaattctgtttttgtaattgtatttttaagggatatgaagctagctaggaagatgaataagaggtgtgagttgtaagggttgggtaagggaatatgagattgtaattggtccaaggcatatcaccttatccatatccacatccaaaatctcctactttactctctctctctctctgacaaccccaacacttgtattgtctcaagcaacc

SEQ ID NO: 4 - DNA, 740 bp, Glycine max
gcacacaactctatcttcatcatcatcatcccccgtgcttcctttatatgctatatattctcatgtgatatcatgtacctattgtcaattttattatgccacaaatattgcttaaactctgtaccttaattttacacttctttttcgctattttggtgattattatttgtgccaactgcatggtttggattaatattgatttgcttcagcttcatccaacttatgctagagtagggaatagtgatagtcatactcaaaccaaacgaggataggttgcgtaaatagtgaaatctgaaatctcgagctgaagtgagaattttgtgatcttcagtgaattgagtattaatattttatatcaaaaaggcgcgttaaagtaagatataatcgtcagggagactgttcacgttctacaagcaatttagtcgttactgcgtgctttttaacttcagattgtgagaagggactggtcatttttttaactatattgtatgattgcatggtatgaaagtttgaaagactaaaaacatgattcaatcgtatatattgaatttgaatcaaacaataaattcgggacacattcaaattaacctctgggctgaattagtgggacgggagaatcatggtcaaccctagaagaaaaaagggcttgataagacaacggaccaggtgagccatagttcaaaattgcagcaacttaaccagcttccaaaccaaatccccagacctgaatccgctgagag

SEQ ID NO: 5 - DNA, 897 bp, Glycine max
gcacacaactctatcttcatcatcatcatcccccgtgcttcctttatatgctatatattctcatgtgatatcatgtacctattgtcaattttattatgccacaaatattgcttaaactctgtaccttaattttacacttctttttcgctattttggtgattattatttgtgccaactgcatggtttggattaatattgatttgcttcagcttcatccaacttatgctagagtagggaatagtgatagtcatactcaaaccaaacgaggataggttgcgtaaatagtgaaatctgaaatctcgagctgaagtgagaattttgtgatcttcagtgaattgagtattaatattttatatcaaaaaggcgcgttaaagtaagatataatcgtcagggagactgttcacgttctacaagcaatttagtcgttactgcgtgctttttaacttcagattgtgagaagggactggtcatttttttaactatattgtatgattgcatggtatgaaagtttgaaagactaaaaacatgattcaatcgtatatattgaatttgaatcaaacaataaattcgggacacattcaaattaacctctgggctgaattagtgggacgggagaatcatggtcaaccctagaagaaaaaagggcttgataagacaacggaccaggtgagccatagttcaaaattgcagcaacttaaccagcttccaaaccaaatccccagacctgaatccgctgagagtttgagtttgaggaaacttaattatgtgaatttgagtttaatagatactatatatgtactattatagtgtaaacattgttaatcagttataaattatttttatatgattttttaagtaattaatataaaaatcaagaaatatataatatacaataat

SEQ ID NO: 6 - DNA, 1416 bp, Artificial Sequence
  Synthetic GmAct7-2 promoter and 5'UTR from Glyma06g15520
aacaccagtatgacgaggtcgaccaacaatactgggaaacacagccctaggagcatcgtcacagcaaatcctgcctgtacacagatgatcatttaaataaattgagcaataatgaaaccaagactaaatagatgcaattacactaacaagaaactgcaaagtactaaccttcaccattccagttccattgtcacaaacaaggggttgaatatcctcagcatcagccattttttaccaaactacagtacgcatacaataaattgtcagtaccaccaagtttgaatagacaatctacagaacccagccatttacagactttgagggtttacttcaaactctctttttctacacaagacagcatcatagtatatataacacacaaaatcaataggaaagaaaacaaggaaaaaaaataattcagtattatacaatctacttagaaataaaacagtaacaaatgtacataaacagataaaggagccgatcctgtgcattttttaaatgaaactgccaaaattaatagatgaatagaaaacgtccattaggacaccagctaaaatctcagaagtcctctgacacagcatatcttaagttcccaaaccaaatgatcttctactaagaaagatcaatgaggaaaaaaataaagccaaaaaagtgataaaaaaaacagatcagaccataaatccatccaacaccagattatgtaatcgatggctatccacatttcagaataagtaaaggtacagttcaaaaagttcgaagatctctgctatagaagatcggaactgtgatatgtcatttccaccactaaaactacagatcgccacaatctactacatttcattcagtatagatcaggtagtacgaatataaataatcagatacaaaacatccagatatgattttgatgaggtaggtaacaatcttatctcacacagatttaaaaagaaaaacataaaaaagagtactactatggaacaaatctaagaataaacattcgagattgcaaaaagcgctgaatcaaagagcaaaaggaaacgtactttgcatcaaagttatgatgtgagagattaagatgaataccttgtgtgagaagaagaagatggcttagcactcactcacacacacacacactctctctctctccggtgcttgagggctacagaaagaggaaagaggaatgagaagagagaaggggagaaggagagggggtatatatatgcggaaagagagagtgtgtcgttggtgtgagagtgagagtgtaatgtaatgtatttgaaattggaattgaggttgggaccaaaaattgaaattgaaggactggagagagagggaatcatttcgaccacgagaaaagagggatagggtgactggatgacagccttttctttttcatttcacacctttctacccttt

SEQ ID NO: 7 - DNA, 1170 bp, Artificial Sequence
  Synthetic GmGAPC2 promoter and 5' UTR from Glyma0618110
cccaaataactgctaattagtatgaataggataggattagtacaatctattgcaggaaagtatgtgttcatgttttattagacaaaaattaaacaaaattttaaaataaaaaacagaggaaatcatgccttggcttggtaacttactatcttctggtccttcatatgataaacaaacagtgtttttttcccctaatcataagaatcatataattatttttaaatgtattaataactatttttttatatctttaatttgttgtgaagtcttttaatgatcactcattattcatgaaagtatatacagttaatgaactattaataatataacttattctcatcggttaacaagtatttttcatgtattatgagtagtgatattatatgtaaccacttcttatatccattgattttatggatatttttaaaataaaatttgaatttatattagtattaattaaaagtaactactttaatcatttttatttgtcttgattatttaatcttatggttttcatttgtgatgatgatcaaagatagtatgatagtatgattttgttatatttgtgcaacacttagttatgtttaataattttttttaaaaaaatataaatatattgaaaaggtcatatgcaagcggtagcctcacccaagaataattaaaatagacccaaattctctgaataaatagacctaaatactccatgaatgtgtttcattgtttgttatttgatgttcatcaaatatcaaatataattaaagctcatcatattctcgtacagtatagtattagtattatatcctgctcactaaaccaaacatctaagaataaccttatttcatttagaaaaaaaacccaagtaaaattgaaaaaagaatcaaaacaataaaaagagagaaaagcgaatggaatattcgcatatctgttggcgtgaaacagaaaccacaaaaaaaacggtacagcgtagtagtccttggcaaagcatcacgagtcacaaggcggtcccgtaggagtcacgcacttcacttggcccatttacctgtcattgcggtcttttactcttctcaataccttattaaaaccctatctcactcactcactcacaccgttccatttctcaacaacttctgctacttcctactccaaccgcacttctgctccgcaattatc

SEQ ID NO: 8 - DNA, 632 bp, Glycine max
aggtgggataggattggagggtatattcggagctgtgatgtatcatatattgtgtggcatccctctggatgtggcgggcacagaattgatgagaagcatttttcaccttggaattcatcaatgtcttcgaaagtaggttgtctgtagcaaaggagtgattgtgaatgcttattttattttctatgtatcctttttcagagttcacattttttttggccttcggaacattaatgtgaatgtctatagctacatgtatcgagaattttatataagattgtcagttcgcactcaaattatcaaattttagtttattcatgaatcacttgcccgatatttgagtgtgctataggcatgaagacacacttaaaagttgtaatggtgaggatacctgcacgatccctggtttaccaggagtccaagggaagggaaaatatctaaatactctaattttgctatcggttaaatttaattttaatattttttagtattgagtttattaatgtgtatgattatgctctgttacgtgttatgtttttagttgagtaaataatttcacaagaatttcagataacaagaataattttacattcaaacctagtggatacacgatatatgaatgaaaagaatattgt

SEQ ID NO: 9 - DNA, 525 bp, Glycine max
ggtgttacttcaaagtagcttgtcttcacattattaccgtatgtttatgtttagctgcgatttagtgtcttgctcgagcaaaaaatgagaggtctgaataaatcggtttctgaaaccagtggtgttacttgttggaggagcattagctcttttttggacttttgatgttttctcttgtggagggggatcgagtttttggatttttatatactcgctgatgtacttggcttgaatacttgctaatgtacttgttattgattgttatagtagatatttgtccgtcctttttttcatttgtggttctcgtatatttgatcctgtttgctttgaatcttggattcgtggtttaaacatttttctgtgcttattttagtccgtatttaaattaacatttttggcttttagttcatattggtttgattggcgtacctgatattcaaaacttaattggttggataagttatactgtaatagtgtgaaagtactttttggaaactgattattccgtgaagttctagataaacg

SEQ ID NO: 10 - DNA, 1686 bp, Artificial Sequence
  The coding sequence of the chimeric RFP/AAD12 reporter gene
atggtgagcaaaggcgaggaacttatcaaagagaacatgcacatgaagctctacatggagggcactgtcaacaatcatcacttcaaatgcacatccgagggagaaggcaagccttatgagggaacccagaccatgaggatcaaagtggttgagggtggaccactcccatttgccttcgacatacttgccactagcttcatgtatggctccagaactttcatcaatcacacacaagggattcccgacttctttaagcagtcttttcctgagggtttcacatgggagcgtgttacaacttacgaagatggtggcgtgttgaccgctactcaagacacttctttgcaagatgggtgtctcatctacaatgtcaagattagaggtgtgaactttccatcaaatggaccagttatgcagaagaaaacccttggatgggaagcaaacaccgagatgctttacccagccgatggtgggcttgaggggaggtctgatatggcactcaagttggttggaggtggccatttgatttgcaacttcaagaccacataccgctcaaagaaacctgctaagaatctcaagatgcctggcgtctactatgtggatcatcgcttggaaaggatcaaggaggcagacaaggaaacctatgtcgaacagcatgaggtggctgttgctcgttactgtgaccttcccagcaagctcggacacaagttgaatctcgccgaggaagcagccgctaaagaggctgcagccaaggaagccgctgcaaaggaggctgccgcaaaagaagccgcagctaaggcagctgccatggctcagaccactctccaaatcacacccactggtgccaccttgggtgccacagtcactggtgttcaccttgccacacttgacgatgctggtttcgctgccctccatgcagcctggcttcaacatgcactcttgatcttccctgggcaacacctcagcaatgaccaacagattacctttgctaaacgctttggagcaattgagaggattggcggaggtgacattgttgccatatccaatgtcaaggcagatggcacagtgcgccagcactctcctgctgagtgggatgacatgatgaaggtcattgtgggcaacatggcctggcacgccgactcaacctacatgccagtcatggctcaaggagctgtgttcagcgcagaagttgtcccagcagttgggggcagaacctgctttgctgacatgagggcagcctacgatgcccttgatgaggcaacccgtgctcttgttcaccaaaggtctgctcgtcactcccttgtgtattctcagagcaagttgggacatgtccaacaggccgggtcagcctacataggttatggcatggacaccactgcaactcctctcagaccattggtcaaggtgcatcctgagactggaaggcccagcctcttgatcggccgccatgcccatgccatccctggcatggatgcagctgaatcagagcgcttccttgaaggacttgttgactgggcctgccaggctcccagagtccatgctcaccaatgggctgctggagatgtggttgtgtgggacaaccgctgtttgctccaccgtgctgagccctgggatttcaagttgccacgtgtgatgtggcactccagactcgctggacgcccagaaactgagggtgctgccttggtttga

SEQ ID NO: 11 - DNA, 3702 bp, Artificial Sequence
  Gene expression casette containing the GmPSID2 promoter - GmPSID 5' UTR - RFP/AAD12 coding sequence - GmPSID2 terminator
caaatggtaaaagaaataaatagttcatactatttttttccaaattttgaaagactttgtgatctcttacagacacaatagcaatcaaatagagaataatcttacgataaaaaaagagaaacaaactcattaaatataataataataactaggataaaataagtttatagccaatttttgttgaatctggtttttagtctatgatatatcatgtaatttagttcctaaaatttatatgaaaaaaaatggttttagtgtatgggttcactcctcaatttttgtacttttcttaacttgagatttagaaaagacactaaaaacaagtattttataaaattctgggacaaaattgtttagtatgaaagtttggaaattagacacaagatttaataaaagtttgtagactaaaaacatattttatctactaaaagtcatcaatttttataacaattatatataattatgtttataatgtaatcttagtaattagatatataaatagataaatgagacttataataataaaaaaaacatataattaactcaagtaataacaattgagaaaaagacatagaaatgtcattcttattatatctattaattagtatacatatttctttgggttagattataattaatgaaaacaaatattagtaaaaagattaatatataataattgataacaaatattattatatttattaataggtgtattttttttactataattattatatattcattaaaaaatttaaggaagggttactaaaagaaaataaaatggttttgagaagagggggggctgatttagatgtctgatttttttaattaaactgtgaagtattcttttagctgagaaacaattctgtttttgtaattgtatttttaagggatatgaagctagctaggaagatgaataagaggtgtgagttgtaagggttgggtaagggaatatgagattgtaattggtccaaggcatatcaccttatccatatccacatccaaaatctcctactttactctctctctctctctgacaaccccaacacttgtattgtctcaagcaaccggatccaaacaatggtgagcaaaggcgaggaacttatcaaagagaacatgcacatgaagctctacatggagggcactgtcaacaatcatcacttcaaatgcacatccgagggagaaggcaagccttatgagggaacccagaccatgaggatcaaagtggttgagggtggaccactcccatttgccttcgacatacttgccactagcttcatgtatggctccagaactttcatcaatcacacacaagggattcccgacttctttaagcagtcttttcctgagggtttcacatgggagcgtgttacaacttacgaagatggtggcgtgttgaccgctactcaagacacttctttgcaagatgggtgtctcatctacaatgtcaagattagaggtgtgaactttccatcaaatggaccagttatgcagaagaaaacccttggatgggaagcaaacaccgagatgctttacccagccgatggtgggcttgaggggaggtctgatatggcactcaagttggttggaggtggccatttgatttgcaacttcaagaccacataccgctcaaagaaacctgctaagaatctcaagatgcctggcgtctactatgtggatcatcgcttggaaaggatcaaggaggcagacaaggaaacctatgtcgaacagcatgaggtggctgttgctcgttactgtgaccttcccagcaagctcggacacaagttgaatctcgccgaggaagcagccgctaaagaggctgcagccaaggaagccgctgcaaaggaggctgccgcaaaagaagccgcagctaaggcagctgccatggctcagaccactctccaaatcacacccactggtgccaccttgggtgccacagtcactggtgttcaccttgccacacttgacgatgctggtttcgctgccctccatgcagcctggcttcaacatgcactcttgatcttccctgggcaacacctcagcaatgaccaacagattacctttgctaaacgctttggagcaattgagaggattggcggaggtgacattgttgccatatccaatgtcaaggcagatggcacagtgcgccagcactctcctgctgagtgggatgacatgatgaaggtcattgtgggcaacatggcctggcacgccgactcaacctacatgccagtcatggctcaaggagctgtgttcagcgcagaagttgtcccagcagttgggggcagaacctgctttgctgacatgagggcagcctacgatgcccttgatgaggcaacccgtgctcttgttcaccaaaggtctgctcgtcactcccttgtgtattctcagagcaagttgggacatgtccaacaggccgggtcagcctacataggttatggcatggacaccactgcaactcctctcagaccattggtcaaggtgcatcctgagactggaaggcccagcctcttgatcggccgccatgcccatgccatccctggcatggatgcagctgaatcagagcgcttccttgaaggacttgttgactgggcctgccaggctcccagagtccatgctcaccaatgggctgctggagatgtggttgtgtgggacaaccgctgtttgctccaccgtgctgagccctgggatttcaagttgccacgtgtgatgtggcactccagactcgctggacgcccagaaactgagggtgctgccttggtttgagtagttagcttaatcacctagagctcggtcaccgagctcgcacacaactctatcttcatcatcatcatcccccgtgcttcctttatatgctatatattctcatgtgatatcatgtacctattgtcaattttattatgccacaaatattgcttaaactctgtaccttaattttacacttctttttcgctattttggtgattattatttgtgccaactgcatggtttggattaatattgatttgcttcagcttcatccaacttatgctagagtagggaatagtgatagtcatactcaaaccaaacgaggataggttgcgtaaatagtgaaatctgaaatctcgagctgaagtgagaattttgtgatcttcagtgaattgagtattaatattttatatcaaaaaggcgcgttaaagtaagatataatcgtcagggagactgttcacgttctacaagcaatttagtcgttactgcgtgctttttaacttcagattgtgagaagggactggtcatttttttaactatattgtatgattgcatggtatgaaagtttgaaagactaaaaacatgattcaatcgtatatattgaatttgaatcaaacaataaattcgggacacattcaaattaacctctgggctgaattagtgggacgggagaatcatggtcaaccctagaagaaaaaagggcttgataagacaacggaccaggtgagccatagttcaaaattgcagcaacttaaccagcttccaaaccaaatccccagacctgaatccgctgagagtttgagtttgaggaaacttaattatgtgaatttgagtttaatagatactatatatgtactattatagtgtaaacattgttaatcagttataaattatttttatatgattttttaagtaattaatataaaaatcaagaaatatataatatacaataat

SEQ ID NO: 12 - DNA, 4584 bp, Artificial Sequence
  Gene expression cassette containing the GFP and PAT reporter/selectable marker genes
gtcgacctgcaggtcaacggatcaggatattcttgtttaagatgttgaactctatggaggtttgtatgaactgatgatctaggaccggataagttcccttcttcatagcgaacttattcaaagaatgttttgtgtatcattcttgttacattgttattaatgaaaaaatattattggtcattggactgaacacgagtgttaaatatggaccaggccccaaataagatccattgatatatgaattaaataacaagaataaatcgagtcaccaaaccacttgccttttttaacgagacttgttcaccaacttgatacaaaagtcattatcctatgcaaatcaataatcatacaaaaatatccaataacactaaaaaattaaaagaaatggataatttcacaatatgttatacgataaagaagttacttttccaagaaattcactgattttataagcccacttgcattagataaatggcaaaaaaaaacaaaaaggaaaagaaataaagcacgaagaattctagaaaatacgaaatacgcttcaatgcagtgggacccacggttcaattattgccaattttcagctccaccgtatatttaaaaaataaaacgataatgctaaaaaaatataaatcgtaacgatcgttaaatctcaacggctggatcttatgacgaccgttagaaattgtggttgtcgacgagtcagtaataaacggcgtcaaagtggttgcagccggcacacacgagtcgtgtttatcaactcaaagcacaaatacttttcctcaacctaaaaataaggcaattagccaaaaacaactttgcgtgtaaacaacgctcaatacacgtgtcattttattattagctattgcttcaccgccttagctttctcgtgacctagtcgtcctcgtcttttcttcttcttcttctataaaacaatacccaaagcttcttcttcacaattcagatttcaatttctcaaaatcttaaaaactttctctcaattctctctaccgtgatcaaggtaaatttctgtgttccttattctctcaaaatcttcgattttgttttcgttcgatcccaatttcgtatatgttctttggtttagattctgttaatcttagatcgaagacgattttctgggtttgatcgttagatatcatcttaattctcgattagggtttcataaatatcatccgatttgttcaaataatttgagttttgtcgaataattactcttcgatttgtgatttctatctagatctggtgttagtttctagtttgtgcgatcgaatttgtcgattaatctgagtttttctgattaacagagatctccatggctcctgccatgaagattgaatgccgcatcactggcaccctcaacggtgtggagtttgaattggttggaggtggagagggcacacctgaacaagggaggatgaccaacaagatgaagtcaactaaaggggctctcaccttcagcccatacttgctttctcatgtcatgggctatggattctaccactttggcacctacccctctggatatgagaaccctttccttcatgccatcaacaatggaggctacacaaacaccagaattgagaagtacgaagatggtggagtcttgcatgtctccttcagctaccgctatgaggctgggagggtcataggagacttcaaagttgtgggcactggattcccagaggactcagtcatcttcactgacaagatcataaggagcaatgccactgttgagcacctccatccaatgggtgacaatgtgcttgttggttcatttgcacgtaccttcagcctcagagatggtggctactattcctttgtggttgattctcacatgcacttcaaatctgcaatccacccctccatcctccagaatgggggtccaatgtttgctttcagacgtgtggaagagttgcacagcaacacagaacttggcattgtggagtaccagcatgccttcaagacacccattgcatttgcttgagtagttagcttaatcacttaggtcaccagcataatttttattaatgtactaaattactgttttgttaaatgcaattttgctttctcgggattttaatatcaaaatctatttagaaatacacaatattttgttgcaggcttgctggagaatcgatctgctatcataaaaattacaaaaaaattttatttgcctcaattattttaggattggtattaaggacgcttaaattatttgtcgggtcactacgcatcattgtgattgagaagatcagcgatacgaaatattcgtagtactatcgataatttatttgaaaattcataagaaaagcaaacgttacatgaattgatgaaacaatacaaagacagataaagccacgcacatttaggatattggccgagattactgaatattgagtaagatcacggaatttctgacaggagcatgtcttcaattcagcccaaatggcagttgaaatactcaaaccgccccatatgcaggagcggatcattcattgtttgtttggttgcctttgccaacatgggagtccaaggttgcggccgcttaattaacttactagtgctagcctcgaggtcgactctgatcatggatgctacgtcacggcagtacaggactatcatcttgaaagtcgattgagcatcgaaacccagctttcttgtacaaagtggttgcggccgcttaattaaatttaaatgtttgggaagctaggccaccgtggcccgcctgcaggggaagcttgtttaaacccagaaggtaattatccaagatgtagcatcaagaatccaatgtttacgggaaaaactatggaagtattatgtaagctcagcaagaagcagatcaatatgcggcacatatgcaacctatgttcaaaaatgaagaatgtacagatacaagatcctatactgccagaatacgaagaagaatacgtagaaattgaaaaagaagaaccaggcgaagaaaagaatcttgaagacgtaagcactgacgacaacaatgaaaagaagaagataaggtcggtgattgtgaaagagacatagaggacacatgtaaggtggaaaatgtaagggcggaaagtaaccttatcacaaaggaatcttatcccccactacttatccttttatatttttccgtgtcatttttgcccttgagttttcctatataaggaaccaagttcggcatttgtgaaaacaagaaaaaatttggtgtaagctattttctttgaagtactgaggatacaacttcagagaaatttgtaagtttgtagatctccatgtctccggagaggagaccagttgagattaggccagctacagcagctgatatggccgcggtttgtgatatcgttaaccattacattgagacgtctacagtgaactttaggacagagccacaaacaccacaagagtggattgatgatctagagaggttgcaagatagatacccttggttggttgctgaggttgagggtgttgtggctggtattgcttacgctgggccctggaaggctaggaacgcttacgattggacagttgagagtactgtttacgtgtcacataggcatcaaaggttgggcctaggatccacattgtacacacatttgcttaagtctatggaggcgcaaggttttaagtctgtggttgctgttataggccttccaaacgatccatctgttaggttgcatgaggctttgggatacacagcccgtggtacattgcgcgcagctggatacaagcatggtggatggcatgatgttggtttttggcaaagggattttgagttgccagctcctccaaggccagttaggccagttacccagatctgactgagcttgagcttatgagcttatgagcttagagctcagatcggcggcaatagcttcttagcgccatcccgggttgatcctatctgtgttgaaatagttgcggtgggcaaggctctctttcagaaagacaggcggccaaaggaacccaaggtgaggtgggctatggctctcagttccttgtggaagcgcttggtctaaggtgcagaggtgttagcggggatgaagcaaaagtgtccgattgtaacaagatatgttgatcctacgtaaggatattaaagtatgtattcatcactaatataatcagtgtattccaatatgtactacgatttccaatgtctttattgtcgccgtatgcaatcggcgtcacaaaataatccccggtgactttcttttaatccaggatgaaataatatgttattataatttttgcgatttggtccgttataggaattgaagtgtgcttgcggtcgccaccactcccatttcataattttacatgtatttgaaaaataaaaatttatggtattcaatttaaacacgtatacttgtaaagaatgatatcttgaaagaaatatagtttaaatatttattgataaaataacaagtcaggtattatagtccaagcaaaaacataaatttattgatgcaagtttaaattcagaaatatttcaataactgattatatcagctggtacattgccgtagatgaaagactgagtgcgatattatggtgtaatacata

SEQ ID NO: 13 - DNA, 22 bp, artificial sequence
  Primer sequence
gaggattagggtttcaacggag

SEQ ID NO: 14 - DNA, 21 bp, Artificial Sequence
  Primer Sequence
gagaattgagctgagacgagg

SEQ ID NO: 15 - DNA, 25 bp, Artificial Sequence
  Probe Sequence
agagaagtttcgacggatttcgggc

SEQ ID NO: 16 - DNA, 29 bp, Artificial Sequence
  Primer Sequence
acaagagtggattgatgatctagagaggt

SEQ ID NO: 17 - DNA, 29 bp, Artificial Sequence
  Primer Sequence
ctttgatgcctatgtgacacgtaaacagt

SEQ ID NO: 18 - DNA, 29 bp, Artificial Sequence
  Probe Sequence
agggtgttgtggctggtattgcttacgct

SEQ ID NO: 19 - DNA, 20 bp, Artificial Sequence
  Primer Sequence
cagagtccatgctcaccaat

SEQ ID NO: 20 - DNA, 19 bp, Artificial Sequence
  Primer Sequence
acgtggcaacttgaaatcc

SEQ ID NO: 21 - DNA, 24 bp, Artificial Sequence
  Probe Sequence
tggagatgtggttgtgtgggacaa

SEQ ID NO: 22 - DNA, 26 bp, artificial sequence
  Primer Sequence
acaagagtggattgatgatctagaga

SEQ ID NO: 23 - DNA, 26 bp, Artificial Sequence
  Primer Sequence
ctttgatgcctatgtgacacgtaaac

SEQ ID NO: 24 - DNA, 29 bp, Artificial Sequence
  Probe Sequence
ccagcgtaagcaataccagccacaacacc

SEQ ID NO: 25 - DNA, 21 bp, Artificial Sequence
  Primer Sequence
cgccgaagtatcgactcaact

SEQ ID NO: 26 - DNA, 19 bp, Artificial Sequence
  Primer Sequence
gcaacgtcggttcgagatg

SEQ ID NO: 27 - DNA, 24 bp, Artificial Sequence
  Probe Sequence
tcagaggtagttggcgtcatcgag